European Patent Application EP 4 706 679 A2, published March 11, 2026. Title: CD6 TARGETED CHIMERIC ANTIGEN RECEPTORS FOR TREATMENT OF CERTAIN AUTOIMMUNE DISORDERS. Applicant: City of Hope. Application EP, filed July 1, 2019. The sequence listing filed with the application follows.

SEQUENCE LISTING (90 sequences)

SEQ ID NO: 1 - protein, 668 aa, Homo sapiens
MWLFFGITGLLTAALSGHPSPAPPDQLNTSSAESELWEPGERLPVRLTNGSSSCSGTVEVRLEASWEPACGALWDSRAAEAVCRALGCGGAEAASQLAPPTPELPPPPAAGNTSVAANATLAGAPALLCSGAEWRLCEVVEHACRSDGRRARVTCAENRALRLVDGGGACAGRVEMLEHGEWGSVCDDTWDLEDAHVVCRQLGCGWAVQALPGLHFTPGRGPIHRDQVNCSGAEAYLWDCPGLPGQHYCGHKEDAGAVCSEHQSWRLTGGADRCEGQVEVHFRGVWNTVCDSEWYPSEAKVLCQSLGCGTAVERPKGLPHSLSGRMYYSCNGEELTLSNCSWRFNNSNLCSQSLAARVLCSASRSLHNLSTPEVPASVQTVTIESSVTVKIENKESRELMLLIPSIVLGILLLGSLIFIAFILLRIKGKYALPVMVNHQHLPTTIPAGSNSYQPVPITIPKEVFMLPIQVQAPPPEDSDSGSDSDYEHYDFSAQPPVALTTFYNSQRHRVTDEEVQQSRFQMPPLEEGLEELHASHIPTANPGHCITDPPSLGPQYHPRSNSESSTSSGEDYCNSPKSKLPPWNPQVFSSERSSFLEQPPNLELAGTQPAFSAGPPADDSSSTSSGEWYQNFQPPPQPPSEEQFGCPGSPSPQPDSTDNDDYDDISAA

SEQ ID NO: 2 - protein, 601 aa, Homo sapiens
MWLFFGITGLLTAALSGHPSPAPPDQLNTSSAESELWEPGERLPVRLTNGSSSCSGTVEVRLEASWEPACGALWDSRAAEAVCRALGCGGAEAASQLAPPTPELPPPPAAGNTSVAANATLAGAPALLCSGAEWRLCEVVEHACRSDGRRARVTCAENRALRLVDGGGACAGRVEMLEHGEWGSVCDDTWDLEDAHVVCRQLGCGWAVQALPGLHFTPGRGPIHRDQVNCSGAEAYLWDCPGLPGQHYCGHKEDAGAVCSEHQSWRLTGGADRCEGQVEVHFRGVWNTVCDSEWYPSEAKVLCQSLGCGTAVERPKGLPHSLSGRMYYSCNGEELTLSNCSWRFNNSNLCSQSLAARVLCSASRSLHNLSTPEVPASVQTVTIESSVTVKIENKESRELMLLIPSIVLGILLLGSLIFIAFILLRIKGKYVFMLPIQVQAPPPEDSDSGSDSDYEHYDFSAQPPVALTTFYNSQRHRVTDEEVQQSRFQMPPLEEGLEELHASHIPTANPGHCITDPPSLGPQYHPRSNSESSTSSGEDYCNSPKSKLPPWNPQVFSSERSSFLEQPPNLELAGTQPAFSGSPSPQPDSTDNDDYDDISAA

SEQ ID NO: 3 - protein, 601 aa, Homo sapiens; identical to SEQ ID NO: 2

SEQ ID NO: 4 - protein, 123 aa, Homo sapiens
MLRLLLALNLFPSIQVTGNKILVKQSPMLVAYDNAVNLSWKHLCPSPLFPGPSKPFWVLVVVGGVLACYSLLVTVAFIIFWVRSKRSRLLHSDYMNMTPRRPGPTRKHYQPYAPPRDFAAYRS

SEQ ID NO: 5 - protein, 101 aa, Homo sapiens
MLRLLLALNLFPSIQVTGKHLCPSPLFPGPSKPFWVLVVVGGVLACYSLLVTVAFIIFWVRSKRSRLLHSDYMNMTPRRPGPTRKHYQPYAPPRDFAAYRS

SEQ ID NO: 6 - protein, 220 aa, Homo sapiens
MLRLLLALNLFPSIQVTGNKILVKQSPMLVAYDNAVNLSCKYSYNLFSREFRASLHKGLDSAVEVCVVYGNYSQQLQVYSKTGFNCDGKLGNESVTFYLQNLYVNQTDIYFCKIEVMYPPPYLDNEKSNGTIIHVKGKHLCPSPLFPGPSKPFWVLVVVGGVLACYSLLVTVAFIIFWVRSKRSRLLHSDYMNMTPRRPGPTRKHYQPYAPPRDFAAYRS

SEQ ID NO: 7 - protein, 41 aa, Homo sapiens
RSKRSRGGHSDYMNMTPRRPGPTRKHYQPYAPPRDFAAYRS

SEQ ID NO: 8 - protein, 41 aa, Homo sapiens
RSKRSRLLHSDYMNMTPRRPGPTRKHYQPYAPPRDFAAYRS

SEQ ID NO: 9 - protein, 458 aa, Homo sapiens
MNRGVPFRHLLLVLQLALLPAATQGKKVVLGKKGDTVELTCTASQKKSIQFHWKNSNQIKILGNQGSFLTKGPSKLNDRADSRRSLWDQGNFPLIIKNLKIEDSDTYICEVEDQKEEVQLLVFGLTANSDTHLLQGQSLTLTLESPPGSSPSVQCRSPRGKNIQGGKTLSVSQLELQDSGTWTCTVLQNQKKVEFKIDIVVLAFQKASSIVYKKEGEQVEFSFPLAFTVEKLTGSGELWWQAERASSSKSWITFDLKNKEVSVKRVTQDPKLQMGKKLPLHLTLPQALPQYAGSGNLTLALEAKTGKLHQEVNLVVMRATQLQKNLTCEVWGPTSPKLMLSLKLENKEAKVSKREKAVWVLNPEAGMWQCLLSDSGQVLLESNIKVLPTWSTPVQPMALIVLGGVAGLLLFIGLGIFFCVRCRHRRRQAERMSQIKRLLSEKKTCQCPHRFQKTCSPI

SEQ ID NO: 10 - protein, 279 aa, Homo sapiens
MPTPLVHPHLPISSPRVSPFPPPAFQKASSIVYKKEGEQVEFSFPLAFTVEKLTGSGELWWQAERASSSKSWITFDLKNKEVSVKRVTQDPKLQMGKKLPLHLTLPQALPQYAGSGNLTLALEAKTGKLHQEVNLVVMRATQLQKNLTCEVWGPTSPKLMLSLKLENKEAKVSKREKAVWVLNPEAGMWQCLLSDSGQVLLESNIKVLPTWSTPVQPMALIVLGGVAGLLLFIGLGIFFCVRCRHRRRQAERMSQIKRLLSEKKTCQCPHRFQKTCSPI

SEQ ID NO: 11 - protein, 185 aa, Homo sapiens
MGKKLPLHLTLPQALPQYAGSGNLTLALEAKTGKLHQEVNLVVMRATQLQKNLTCEVWGPTSPKLMLSLKLENKEAKVSKREKAVWVLNPEAGMWQCLLSDSGQVLLESNIKVLPTWSTPVQPMALIVLGGVAGLLLFIGLGIFFCVRCRHRRRQAERMSQIKRLLSEKKTCQCPHRFQKTCSPI

SEQ ID NO: 12 - protein, 185 aa, Homo sapiens; identical to SEQ ID NO: 11

SEQ ID NO: 13 - protein, 185 aa, Homo sapiens; identical to SEQ ID NO: 11

SEQ ID NO: 14 - protein, 42 aa, Homo sapiens
KRGRKKLLYIFKQPFMRPVQTTQEEDGCSCRFPEEEEGGCEL

SEQ ID NO: 15 - protein, 255 aa, Homo sapiens
MGNSCYNIVATLLLVLNFERTRSLQDPCSNCPAGTFCDNNRNQICSPCPPNSFSSAGGQRTCDICRQCKGVFRTRKECSSTSNAECDCTPGFHCLGAGCSMCEQDCKQGQELTKKGCKDCCFGTFNDQKRGICRPWTNCSLDGKSVLVNGTKERDVVCGPSPADLSPGASSVTPPAPAREPGHSPQIISFFLALTSTALLFLLFFLTLRFSVVKRGRKKLLYIFKQPFMRPVQTTQEEDGCSCRFPEEEEGGCEL

SEQ ID NO: 16 - protein, 199 aa, Homo sapiens
MKSGLWYFFLFCLRIKVLTGEINGSANYEMFIFHNGGVQILCKYPDIVQQFKMQLLKGGQILCDLTKTKGSGNTVSIKSLKFCHSQLSNNSVSFFLYNLDHSHANYYFCNLSIFDPPPFKVTLTGGYLHIYESQLCCQLKFWLPIGCAAFVVVCILGCILICWLTKKKYSSSVHDPNGEYMFMRAVNTAKKSRLTDVTL

SEQ ID NO: 17 - protein, 41 aa, Homo sapiens
AVSLSKMLKKRSPLTTGVYVKMPPTEPECEKQFQPYFIPIN

SEQ ID NO: 18 - DNA, 327 bp, Homo sapiens
  source 1..327: mol_type = other DNA
gacatccaaatgacacaaagtcctagctctctctcagcaagtgttggcgaccgtgtgaccatcacatgtaaagcttcaagggatattcgcagctacctgacttggtaccaacaaaagcccggaaaagcgcctaaaacgcttatttactatgccaccagcctcgcagatggtgtcccctccagattttctggatcgggatcagggcaagattatagtcttacgatatcgagtcttgagtcggacgatactgccacatactactgcttacagcacggggaaagcccattcacattcggaagtggtacgaaactcgagatcaaacgggca

SEQ ID NO: 19 - DNA, 357 bp, Homo sapiens
  source 1..357: mol_type = other DNA
gaagtccaattggtcgagagcggaggtgggcttgttaaaccaggaggcagtttaaaattatcatgtgctgcctcgggtttcaagttctcgcggtatgctatgtcctgggtacgccaagcacctggaaagcgtttagaatgggtggccacaattagtagtggtggttcatatatatattatcccgactccgtcaaaggaaggttcacgatttcaagggacaatgtgaagaacaccctctacttacagatgagtagtctgcgttctgaggataccgctatgtactactgtgctcggagagattacgatctggattatttcgacagctggggtcagggcacactcgttacagtatcctcg

SEQ ID NO: 20 - DNA, 60 bp, Homo sapiens
  source 1..60: mol_type = other DNA
gtccaacttgttgaatcaggtggggggctggtcaaacccgggggctctctgaaactaagt

SEQ ID NO: 21 - DNA, 45 bp, Homo sapiens
  source 1..45: mol_type = other DNA
ttctctcggtacgctatgtcgtgggtcagacaagcgcccggcaaa

SEQ ID NO: 22 - DNA, 57 bp, Homo sapiens
  source 1..57: mol_type = other DNA
cgtgattatgatctagactactttgactcctggggtcaaggtacgctcgtgacggtt

SEQ ID NO: 23 - protein, 22 aa, Homo sapiens
MALIVLGGVAGLLLFIGLGIFF

SEQ ID NO: 24 - DNA, 66 bp, Homo sapiens
  source 1..66: mol_type = other DNA
atggccctgattgtgctggggggcgtcgccggcctcctgcttttcattgggctaggcatcttcttc

SEQ ID NO: 25 - protein, 21 aa, Homo sapiens
IYIWAPLAGTCGVLLLSLVIT

SEQ ID NO: 26 - DNA, 54 bp, Homo sapiens
  source 1..54: mol_type = other DNA
gggtcaacgtcgggcgggggttccggtggaggaagtggaggtggtggaagttct

SEQ ID NO: 27 - DNA, 60 bp, Homo sapiens
  source 1..60: mol_type = other DNA
ggcggcggcggaagtggcggcggcggctcaggcggggggggttctgggggcggcggttca

SEQ ID NO: 28 - protein, 20 aa, Homo sapiens
VQLVESGGGLVKPGGSLKLS

SEQ ID NO: 29 - protein, 15 aa, Homo sapiens
FSRYAMSWVRQAPGK

SEQ ID NO: 30 - protein, 19 aa, Homo sapiens
RDYDLDYFDSWGQGTLVTV

SEQ ID NO: 31 - protein, 38 aa, Homo sapiens
CWLTKKKYSSSVHDPNGEYMFMRAVNTAKKSRLTDVTL

SEQ ID NO: 32 - protein, 42 aa, Homo sapiens
ALYLLRRDQRLPPDAHKPPGGGSFRTPIQEEQADAHSTLAKI

SEQ ID NO: 33 - protein, 97 aa, Homo sapiens
CSRAARGTIGARRTGQPLKEDPSAVPVFSVDYGELDFQWREKTPEPPVPCVPEQTEYATIVFPSGMGTSSPARRGSADGPRSAQPLRPEDGHCSWPL

SEQ ID NO: 34 - protein, 109 aa, Homo sapiens
DIQMTQSPSSLSASVGDRVTITCKASRDIRSYLTWYQQKPGKAPKTLIYYATSLADGVPSRFSGSGSGQDYSLTISSLESDDTATYYCLQHGESPFTFGSGTKLEIKRA

SEQ ID NO: 35 - protein, 119 aa, Homo sapiens
EVQLVESGGGLVKPGGSLKLSCAASGFKFSRYAMSWVRQAPGKRLEWVATISSGGSYIYYPDSVKGRFTISRDNVKNTLYLQMSSLRSEDTAMYYCARRDYDLDYFDSWGQGTLVTVSS

SEQ ID NO: 36 - protein, 18 aa, Homo sapiens
GSTSGGGSGGGSGGGGSS

SEQ ID NO: 37 - protein, 20 aa, Homo sapiens
GGGGSGGGGSGGGGSGGGGS

SEQ ID NO: 38 - protein, 246 aa, Homo sapiens
EVQLVESGGGLVKPGGSLKLSCAASGFKFSRYAMSWVRQAPGKRLEWVATISSGGSYIYYPDSVKGRFTISRDNVKNTLYLQMSSLRSEDTAMYYCARRDYDLDYFDSWGQGTLVTVSSGSTSGGGSGGGSGGGGSSDIQMTQSPSSLSASVGDRVTITCKASRDIRSYLTWYQQKPGKAPKTLIYYATSLADGVPSRFSGSGSGQDYSLTISSLESDDTATYYCLQHGESPFTFGSGTKLEIKRA

SEQ ID NO: 39 - protein, 248 aa, Homo sapiens
EVQLVESGGGLVKPGGSLKLSCAASGFKFSRYAMSWVRQAPGKRLEWVATISSGGSYIYYPDSVKGRFTISRDNVKNTLYLQMSSLRSEDTAMYYCARRDYDLDYFDSWGQGTLVTVSSGGGGSGGGGSGGGGSGGGGSDIQMTQSPSSLSASVGDRVTITCKASRDIRSYLTWYQQKPGKAPKTLIYYATSLADGVPSRFSGSGSGQDYSLTISSLESDDTATYYCLQHGESPFTFGSGTKLEIKRA

SEQ ID NO: 40 - protein, 246 aa, Homo sapiens
DIQMTQSPSSLSASVGDRVTITCKASRDIRSYLTWYQQKPGKAPKTLIYYATSLADGVPSRFSGSGSGQDYSLTISSLESDDTATYYCLQHGESPFTFGSGTKLEIKRAGSTSGGGSGGGSGGGGSSEVQLVESGGGLVKPGGSLKLSCAASGFKFSRYAMSWVRQAPGKRLEWVATISSGGSYIYYPDSVKGRFTISRDNVKNTLYLQMSSLRSEDTAMYYCARRDYDLDYFDSWGQGTLVTVSS

SEQ ID NO: 41 - protein, 248 aa, Homo sapiens
DIQMTQSPSSLSASVGDRVTITCKASRDIRSYLTWYQQKPGKAPKTLIYYATSLADGVPSRFSGSGSGQDYSLTISSLESDDTATYYCLQHGESPFTFGSGTKLEIKRAGGGGSGGGGSGGGGSGGGGSEVQLVESGGGLVKPGGSLKLSCAASGFKFSRYAMSWVRQAPGKRLEWVATISSGGSYIYYPDSVKGRFTISRDNVKNTLYLQMSSLRSEDTAMYYCARRDYDLDYFDSWGQGTLVTVSS

SEQ ID NO: 42 - DNA, 738 bp, Homo sapiens
  source 1..738: mol_type = other DNA
gaagtccaattggtcgagagcggaggtgggcttgttaaaccaggaggcagtttaaaattatcatgtgctgcctcgggtttcaagttctcgcggtatgctatgtcctgggtacgccaagcacctggaaagcgtttagaatgggtggccacaattagtagtggtggttcatatatatattatcccgactccgtcaaaggaaggttcacgatttcaagggacaatgtgaagaacaccctctacttacagatgagtagtctgcgttctgaggataccgctatgtactactgtgctcggagagattacgatctggattatttcgacagctggggtcagggcacactcgttacagtatcctcggggtcaacgtcgggcgggggttccggtggaggaagtggaggtggtggaagttctgacatccaaatgacacaaagtcctagctctctctcagcaagtgttggcgaccgtgtgaccatcacatgtaaagcttcaagggatattcgcagctacctgacttggtaccaacaaaagcccggaaaagcgcctaaaacgcttatttactatgccaccagcctcgcagatggtgtcccctccagattttctggatcgggatcagggcaagattatagtcttacgatatcgagtcttgagtcggacgatactgccacatactactgcttacagcacggggaaagcccattcacattcggaagtggtacgaaactcgagatcaaacgggca

SEQ ID NO: 43 - DNA, 744 bp, Homo sapiens
  source 1..744: mol_type = other DNA
gaagtccaattggtcgagagcggaggtgggcttgttaaaccaggaggcagtttaaaattatcatgtgctgcctcgggtttcaagttctcgcggtatgctatgtcctgggtacgccaagcacctggaaagcgtttagaatgggtggccacaattagtagtggtggttcatatatatattatcccgactccgtcaaaggaaggttcacgatttcaagggacaatgtgaagaacaccctctacttacagatgagtagtctgcgttctgaggataccgctatgtactactgtgctcggagagattacgatctggattatttcgacagctggggtcagggcacactcgttacagtatcctcgggcggcggcggaagtggcggcggcggctcaggcggggggggttctgggggcggcggttcagacatccaaatgacacaaagtcctagctctctctcagcaagtgttggcgaccgtgtgaccatcacatgtaaagcttcaagggatattcgcagctacctgacttggtaccaacaaaagcccggaaaagcgcctaaaacgcttatttactatgccaccagcctcgcagatggtgtcccctccagattttctggatcgggatcagggcaagattatagtcttacgatatcgagtcttgagtcggacgatactgccacatactactgcttacagcacggggaaagcccattcacattcggaagtggtacgaaactcgagatcaaacgggca

SEQ ID NO: 44 - DNA, 738 bp, Homo sapiens
  source 1..738: mol_type = other DNA
gacatccaaatgacacaaagtcctagctctctctcagcaagtgttggcgaccgtgtgaccatcacatgtaaagcttcaagggatattcgcagctacctgacttggtaccaacaaaagcccggaaaagcgcctaaaacgcttatttactatgccaccagcctcgcagatggtgtcccctccagattttctggatcgggatcagggcaagattatagtcttacgatatcgagtcttgagtcggacgatactgccacatactactgcttacagcacggggaaagcccattcacattcggaagtggtacgaaactcgagatcaaacgggcagggtcaacgtcgggcgggggttccggtggaggaagtggaggtggtggaagttctgaagtccaattggtcgagagcggaggtgggcttgttaaaccaggaggcagtttaaaattatcatgtgctgcctcgggtttcaagttctcgcggtatgctatgtcctgggtacgccaagcacctggaaagcgtttagaatgggtggccacaattagtagtggtggttcatatatatattatcccgactccgtcaaaggaaggttcacgatttcaagggacaatgtgaagaacaccctctacttacagatgagtagtctgcgttctgaggataccgctatgtactactgtgctcggagagattacgatctggattatttcgacagctggggtcagggcacactcgttacagtatcctcg

SEQ ID NO: 45 - DNA, 744 bp, Homo sapiens
  source 1..744: mol_type = other DNA
gacatccaaatgacacaaagtcctagctctctctcagcaagtgttggcgaccgtgtgaccatcacatgtaaagcttcaagggatattcgcagctacctgacttggtaccaacaaaagcccggaaaagcgcctaaaacgcttatttactatgccaccagcctcgcagatggtgtcccctccagattttctggatcgggatcagggcaagattatagtcttacgatatcgagtcttgagtcggacgatactgccacatactactgcttacagcacggggaaagcccattcacattcggaagtggtacgaaactcgagatcaaacgggcaggcggcggcggaagtggcggcggcggctcaggcggggggggttctgggggcggcggttcagaagtccaattggtcgagagcggaggtgggcttgttaaaccaggaggcagtttaaaattatcatgtgctgcctcgggtttcaagttctcgcggtatgctatgtcctgggtacgccaagcacctggaaagcgtttagaatgggtggccacaattagtagtggtggttcatatatatattatcccgactccgtcaaaggaaggttcacgatttcaagggacaatgtgaagaacaccctctacttacagatgagtagtctgcgttctgaggataccgctatgtactactgtgctcggagagattacgatctggattatttcgacagctggggtcagggcacactcgttacagtatcctcg

SEQ ID NO: 46 - protein, 235 aa, Homo sapiens
MALPVTALLLPLALLLHAARPSQFRVSPLDRTWNLGETVELKCQVLLSNPTSGCSWLFQPRGAAASPTFLLYLSQNKPKAAEGLDTQRFSGKRLGDTFVLTLSDFRRENEGYYFCSALSNSIMYFSHFVPVFLPAKPTTTPAPRPPTPAPTIASQPLSLRPEACRPAAGGAVHTRGLDFACDIYIWAPLAGTCGVLLLSLVITLYCNHRNRRRVCKCPRPVVKSGDKPSLSARYV

SEQ ID NO: 47 - protein, 198 aa, Homo sapiens
MALPVTALLLPLALLLHAARPSQFRVSPLDRTWNLGETVELKCQVLLSNPTSGCSWLFQPRGAAASPTFLLYLSQNKPKAAEGLDTQRFSGKRLGDTFVLTLSDFRRENEGYYFCSALSNSIMYFSHFVPVFLPAKPTTTPAPRPPTPAPTIASQPLSLRPEACRPAAGGAGNRRRVCKCPRPVVKSGDKPSLSARYV

SEQ ID NO: 48 - protein, 235 aa, Homo sapiens; identical to SEQ ID NO: 46

SEQ ID NO: 49 - protein, 246 aa, Homo sapiens
MRPRLWLLLAAQLTVLHGNSVLQQTPAYIKVQTNKMVMLSCEAKISLSNMRIYWLRQRQAPSSDSHHEFLALWDSAKGTIHGEEVEQEKIAVFRDASRFILNLTSVKPEDSGIYFCMIVGSPELTFGKGTQLSVVDFLPTTAQPTKKSTLKKRVCRLPRPETQKGPLCSPITLGLLVAGVLVLLVSLGVAIHLCCRRRRARLRFMKQKFNIVCLKISGFTTCCCFQILQMSREYGFGVLLQKDIGQ

SEQ ID NO: 50 - protein, 198 aa, Homo sapiens
MRPRLWLLLAAQLTVLHGNSVLQQTPAYIKVQTNKMVMLSCEAKISLSNMRIYWLRQRQAPSSDSHHEFLALWDSAKGTIHGEEVEQEKIAVFRDASRFILNLTSVKPEDSGIYFCMIVGSPELTFGKGTQLSVVDFLPTTAQPTKKSTLKKRVCRLPRPETQKGLKGKVYQEPLSPNACMDTTAILQPHRSCLTHGS

SEQ ID NO: 51 - protein, 243 aa, Homo sapiens
MRPRLWLLLAAQLTVLHGNSVLQQTPAYIKVQTNKMVMLSCEAKISLSNMRIYWLRQRQAPSSDSHHEFLALWDSAKGTIHGEEVEQEKIAVFRDASRFILNLTSVKPEDSGIYFCMIVGSPELTFGKGTQLSVVDFLPTTAQPTKKSTLKKRVCRLPRPETQKGPLCSPITLGLLVAGVLVLLVSLGVAIHLCCRRRRARLRFMKQPQGEGISGTFVPQCLHGYYSNTTTSQKLLNPWILKT

SEQ ID NO: 52 - protein, 213 aa, Homo sapiens
MRPRLWLLLAAQLTVLHGNSVLQQTPAYIKVQTNKMVMLSCEAKISLSNMRIYWLRQRQAPSSDSHHEFLALWDSAKGTIHGEEVEQEKIAVFRDASRFILNLTSVKPEDSGIYFCMIVGSPELTFGKGTQLSVVDFLPTTAQPTKKSTLKKRVCRLPRPETQKGRRRRARLRFMKQPQGEGISGTFVPQCLHGYYSNTTTSQKLLNPWILKT

SEQ ID NO: 53 - protein, 221 aa, Homo sapiens
MRPRLWLLLAAQLTVLHGNSVLQQTPAYIKVQTNKMVMLSCEAKISLSNMRIYWLRQRQAPSSDSHHEFLALWDSAKGTIHGEEVEQEKIAVFRDASRFILNLTSVKPEDSGIYFCMIVGSPELTFGKGTQLSVVDFLPTTAQPTKKSTLKKRVCRLPRPETQKGPLCSPITLGLLVAGVLVLLVSLGVAIHLCCRRRRARLRFMKQLRLHPLEKCSRMDY

SEQ ID NO: 54 - protein, 210 aa, Homo sapiens
MRPRLWLLLAAQLTVLHGNSVLQQTPAYIKVQTNKMVMLSCEAKISLSNMRIYWLRQRQAPSSDSHHEFLALWDSAKGTIHGEEVEQEKIAVFRDASRFILNLTSVKPEDSGIYFCMIVGSPELTFGKGTQLSVVDFLPTTAQPTKKSTLKKRVCRLPRPETQKGPLCSPITLGLLVAGVLVLLVSLGVAIHLCCRRRRARLRFMKQFYK

SEQ ID NO: 55 - protein, 163 aa, Homo sapiens
MKWKALFTAAILQAQLPITEAQSFGLLDPKLCYLLDGILFIYGVILTALFLRVKFSRSADAPAYQQGQNQLYNELNLGRREEYDVLDKRRGRDPEMGGKPRRKNPQEGLYNELQKDKMAEAYSEIGMKGERRRGKGHDGLYQGLSTATKDTYDALHMQALPPR

SEQ ID NO: 56 - protein, 164 aa, Homo sapiens
MKWKALFTAAILQAQLPITEAQSFGLLDPKLCYLLDGILFIYGVILTALFLRVKFSRSADAPAYQQGQNQLYNELNLGRREEYDVLDKRRGRDPEMGGKPQRRKNPQEGLYNELQKDKMAEAYSEIGMKGERRRGKGHDGLYQGLSTATKDTYDALHMQALPPR

SEQ ID NO: 57 - protein, 123 aa, Homo sapiens; identical to SEQ ID NO: 4

SEQ ID NO: 58 - protein, 101 aa, Homo sapiens; identical to SEQ ID NO: 5

SEQ ID NO: 59 - protein, 220 aa, Homo sapiens; identical to SEQ ID NO: 6

SEQ ID NO: 60 - protein, 277 aa, Homo sapiens
MCVGARRLGRGPCAALLLLGLGLSTVTGLHCVGDTYPSNDRCCHECRPGNGMVSRCSRSQNTVCRPCGPGFYNDVVSSKPCKPCTWCNLRSGSERKQLCTATQDTVCRCRAGTQPLDSYKPGVDCAPCPPGHFSPGDNQACKPWTNCTLAGKHTLQPASNSSDAICEDRDPPATQPQETQGPPARPITVQPTEAWPRTSQGPSTRPVEVPGGRAVAAILGLGLVLGLLGPLAILLALYLLRRDQRLPPDAHKPPGGGSFRTPIQEEQADAHSTLAKI

SEQ ID NO: 61 - protein, 174 aa, Homo sapiens
MACLGFQRHKAQLNLATRTWPCTLLFFLLFIPVFCKAMHVAQPAVVLASSRGIASFVCEYASPGKATEVRVTVLRQADSQVTEVCAATYMMGNELTFLDDSICTGTSSGNQVNLTIQGLRAMDTGLYICKVELMYPPPYYLGIGNGTQIYVIAKEKKPSYNRGLCENAPNRARM

SEQ ID NO: 62 - protein, 223 aa, Homo sapiens
MACLGFQRHKAQLNLATRTWPCTLLFFLLFIPVFCKAMHVAQPAVVLASSRGIASFVCEYASPGKATEVRVTVLRQADSQVTEVCAATYMMGNELTFLDDSICTGTSSGNQVNLTIQGLRAMDTGLYICKVELMYPPPYYLGIGNGTQIYVIDPEPCPDSDFLLWILAAVSSGLFFYSFLLTAVSLSKMLKKRSPLTTGVYVKMPPTEPECEKQFQPYFIPIN

SEQ ID NO: 63 - protein, 288 aa, Homo sapiens
MQIPQAPWPVVWAVLQLGWRPGWFLDSPDRPWNPPTFSPALLVVTEGDNATFTCSFSNTSESFVLNWYRMSPSNQTDKLAAFPEDRSQPGQDCRFRVTQLPNGRDFHMSVVRARRNDSGTYLCGAISLAPKAQIKESLRAELRVTERRAEVPTAHPSPSPRPAGQFQTLVVGVVGGLLGSLVLLVWVLAVICSRAARGTIGARRTGQPLKEDPSAVPVFSVDYGELDFQWREKTPEPPVPCVPEQTEYATIVFPSGMGTSSPARRGSADGPRSAQPLRPEDGHCSWPL

SEQ ID NO: 64 - protein, 241 aa, Homo sapiens
MAQHGAMGAFRALCGLALLCALSLGQRPTGGPGCGPGRLLLGTGTDARCCRVHTTRCCRDYPGEECCSEWDCMCVQPEFHCGDPCCTTCRHHPCPPGQGVQSQGKFSFGFQCIDCASGTFSGGHEGHCKPWTDCTQFGFLTVFPGNKTHNAVCVPGSPPAEPLGWLTVVLLAVAACVLLLTSAQLGLHIWQLRSQCMWPRETQLLLEVPPSTEDARSCQFPEEERGERSAEEKGRLGDLWV

SEQ ID NO: 65 - protein, 255 aa, Homo sapiens
MAQHGAMGAFRALCGLALLCALSLGQRPTGGPGCGPGRLLLGTGTDARCCRVHTTRCCRDYPGEECCSEWDCMCVQPEFHCGDPCCTTCRHHPCPPGQGVQSQGKFSFGFQCIDCASGTFSGGHEGHCKPWTDCCWRCRRRPKTPEAASSPRKSGASDRQRRRGGWETCGCEPGRPPGPPTAASPSPGAPQAAGALRSALGRALLPWQQKWVQEGGSDQRPGPCSSAAAAGPCRRERETQSWPPSSLAGPDGVGS

SEQ ID NO: 66 - protein, 234 aa, Homo sapiens
MAQHGAMGAFRALCGLALLCALSLGQRPTGGPGCGPGRLLLGTGTDARCCRVHTTRCCRDYPGEECCSEWDCMCVQPEFHCGDPCCTTCRHHPCPPGQGVQSQGKFSFGFQCIDCASGTFSGGHEGHCKPWTDCTQFGFLTVFPGNKTHNAVCVPGSPPAEPLGWLTVVLLAVAACVLLLTSAQLGLHIWQLRKTQLLLEVPPSTEDARSCQFPEEERGERSAEEKGRLGDLWV

SEQ ID NO: 67 - protein, 57 aa, Homo sapiens
QLGLHIWQLRSQCMWPRETQLLLEVPPSTEDARSCQFPEEERGERSAEEKGRLGDLW

SEQ ID NO: 68 - protein, 118 aa, Homo sapiens
EVQLVESGGGLVKPGGSLKLSCAASGFKFSRYAMSWVRQTPEKRLEWVATISSGGSYIYYPDSVKGRFTISRDNVKNTLYLQMSSLRSEDTAMYYCARRDYDLDYFDSWGQGTTLTVS

SEQ ID NO: 69 - protein, 109 aa, Homo sapiens
DIKMTQSPSSMYASLGERVTITCKASRDIRSYLTWYQQKPWKSPKTLIYYATSLADGVPSRFSGSGSGQDYSLTISSLESDDTATYYCLQHGESPFTFGSGTKLEIKRA

SEQ ID NO: 70 - protein, 22 aa, Homo sapiens
MLLLVTSLLLCELPHPAFLLIP

SEQ ID NO: 71 - protein, 24 aa, Homo sapiens
LEGGGEGRGSLLTCGDVEENPGPR

SEQ ID NO: 72 - skipped

SEQ ID NO: 73 - protein, 323 aa, Homo sapiens
MPPPRLLFFLLFLTPMEVRPEEPLVVKVEEGDNAVLQCLKGTSDGPTQQLTWSRESPLKPFLKLSLGLPGLGIHMRPLAIWLFIFNVSQQMGGFYLCQPGPPSEKAWQPGWTVNVEGSGELFRWNVSDLGGLGCGLKNRSSEGPSSPSGKLMSPKLYVWAKDRPEIWEGEPPCVPPRDSLNQSLSQDLTMAPGSTLWLSCGVPPDSVSRGPLSWTHVHPKGPKSLLSLELKDDRPARDMWVMETGLLLPRATAQDAGKYYCHRGNLTMSFHLEITARPVLWHWLLRTGGWKVSAVTLAYLIFCLCSLVGILHLQRALVLRRKR

SEQ ID NO: 74 - skipped

SEQ ID NO: 75 - protein, 68 aa, Homo sapiens
IQMTQSPSSLSASVGDRVTITCKASRDIRSYLTWYQQKPGKAPKTLIYYATSLADGVPSRFSGSGSGQ

SEQ ID NO: 76 - protein, 32 aa, Homo sapiens
DIQMTQSPSSLSASVGDRVTITCKASRDIRSY

SEQ ID NO: 77 - protein, 65 aa, Homo sapiens
LTWYQQKPGKAPKTLIYYATSLADGVPSRFSGSGSGQDYSLTISSLESDDTATYYCLQHGESPFT

SEQ ID NO: 78 - protein, 12 aa, Homo sapiens
FGSGTKLEIKRA

SEQ ID NO: 79 - protein, 35 aa, Homo sapiens
EVQLVESGGGLVKPGGSLKLSCAASGFKFSRYAMS

SEQ ID NO: 80 - protein, 20 aa, Homo sapiens
WVRQAPGKRLEWVATISSGG

SEQ ID NO: 81 - protein, 53 aa, Homo sapiens
SYIYYPDSVKGRFTISRDNVKNTLYLQMSSLRSEDTAMYYCARRDYDLDYFDS

SEQ ID NO: 82 - protein, 11 aa, Homo sapiens
WGQGTLVTVSS

SEQ ID NO: 83 - protein, 653 aa, Homo sapiens
EVQLVESGGGLVKPGGSLKLSCAASGFKFSRYAMSWVRQAPGKRLEWVATISSGGSYIYYPDSVKGRFTISRDNVKNTLYLQMSSLRSEDTAMYYCARRDYDLDYFDSWGQGTLVTVSSGSTSGGGSGGGSGGGGSSDIQMTQSPSSLSASVGDRVTITCKASRDIRSYLTWYQQKPGKAPKTLIYYATSLADGVPSRFSGSGSGQDYSLTISSLESDDTATYYCLQHGESPFTFGSGTKLEIKRAESKYGPPCPPCPAPEFEGGPSVFLFPPKPKDTLMISRTPEVTCVVVDVSQEDPEVQFNWYVDGVEVHNAKTKPREEQFQSTYRVVSVLTVLHQDWLNGKEYKCKVSNKGLPSSIEKTISKAKGQPREPQVYTLPPSQEEMTKNQVSLTCLVKGFYPSDIAVEWESNGQPENNYKTTPPVLDSDGSFFLYSRLTVDKSRWQEGNVFSCSVMHEALHNHYTQKSLSLSLGKMALIVLGGVAGLLLFIGLGIFFAVSLSKMLKKRSPLTTGVYVKMPPTEPECEKQFQPYFIPINGGGRVKFSRSADAPAYQQGQNQLYNELNLGRREEYDVLDKRRGRDPEMGGKPRRKNPQEGLYNELQKDKMAEAYSEIGMKGERRRGKGHDGLYQGLSTATKDTYDALHMQALPPR

SEQ ID NO: 84 - protein, 675 aa, Homo sapiens
MLLLVTSLLLCELPHPAFLLIPEVQLVESGGGLVKPGGSLKLSCAASGFKFSRYAMSWVRQAPGKRLEWVATISSGGSYIYYPDSVKGRFTISRDNVKNTLYLQMSSLRSEDTAMYYCARRDYDLDYFDSWGQGTLVTVSSGSTSGGGSGGGSGGGGSSDIQMTQSPSSLSASVGDRVTITCKASRDIRSYLTWYQQKPGKAPKTLIYYATSLADGVPSRFSGSGSGQDYSLTISSLESDDTATYYCLQHGESPFTFGSGTKLEIKRAESKYGPPCPPCPAPEFEGGPSVFLFPPKPKDTLMISRTPEVTCVVVDVSQEDPEVQFNWYVDGVEVHNAKTKPREEQFQSTYRVVSVLTVLHQDWLNGKEYKCKVSNKGLPSSIEKTISKAKGQPREPQVYTLPPSQEEMTKNQVSLTCLVKGFYPSDIAVEWESNGQPENNYKTTPPVLDSDGSFFLYSRLTVDKSRWQEGNVFSCSVMHEALHNHYTQKSLSLSLGKMALIVLGGVAGLLLFIGLGIFFAVSLSKMLKKRSPLTTGVYVKMPPTEPECEKQFQPYFIPINGGGRVKFSRSADAPAYQQGQNQLYNELNLGRREEYDVLDKRRGRDPEMGGKPRRKNPQEGLYNELQKDKMAEAYSEIGMKGERRRGKGHDGLYQGLSTATKDTYDALHMQALPPR

SEQ ID NO: 85 - protein, 653 aa, Homo sapiens
DIQMTQSPSSLSASVGDRVTITCKASRDIRSYLTWYQQKPGKAPKTLIYYATSLADGVPSRFSGSGSGQDYSLTISSLESDDTATYYCLQHGESPFTFGSGTKLEIKRAGSTSGGGSGGGSGGGGSSEVQLVESGGGLVKPGGSLKLSCAASGFKFSRYAMSWVRQAPGKRLEWVATISSGGSYIYYPDSVKGRFTISRDNVKNTLYLQMSSLRSEDTAMYYCARRDYDLDYFDSWGQGTLVTVSSESKYGPPCPPCPAPEFEGGPSVFLFPPKPKDTLMISRTPEVTCVVVDVSQEDPEVQFNWYVDGVEVHNAKTKPREEQFQSTYRVVSVLTVLHQDWLNGKEYKCKVSNKGLPSSIEKTISKAKGQPREPQVYTLPPSQEEMTKNQVSLTCLVKGFYPSDIAVEWESNGQPENNYKTTPPVLDSDGSFFLYSRLTVDKSRWQEGNVFSCSVMHEALHNHYTQKSLSLSLGKMALIVLGGVAGLLLFIGLGIFFAVSLSKMLKKRSPLTTGVYVKMPPTEPECEKQFQPYFIPINGGGRVKFSRSADAPAYQQGQNQLYNELNLGRREEYDVLDKRRGRDPEMGGKPRRKNPQEGLYNELQKDKMAEAYSEIGMKGERRRGKGHDGLYQGLSTATKDTYDALHMQALPPR

SEQ ID NO: 86 - protein, 675 aa, Homo sapiens
MLLLVTSLLLCELPHPAFLLIPDIQMTQSPSSLSASVGDRVTITCKASRDIRSYLTWYQQKPGKAPKTLIYYATSLADGVPSRFSGSGSGQDYSLTISSLESDDTATYYCLQHGESPFTFGSGTKLEIKRAGSTSGGGSGGGSGGGGSSEVQLVESGGGLVKPGGSLKLSCAASGFKFSRYAMSWVRQAPGKRLEWVATISSGGSYIYYPDSVKGRFTISRDNVKNTLYLQMSSLRSEDTAMYYCARRDYDLDYFDSWGQGTLVTVSSESKYGPPCPPCPAPEFEGGPSVFLFPPKPKDTLMISRTPEVTCVVVDVSQEDPEVQFNWYVDGVEVHNAKTKPREEQFQSTYRVVSVLTVLHQDWLNGKEYKCKVSNKGLPSSIEKTISKAKGQPREPQVYTLPPSQEEMTKNQVSLTCLVKGFYPSDIAVEWESNGQPENNYKTTPPVLDSDGSFFLYSRLTVDKSRWQEGNVFSCSVMHEALHNHYTQKSLSLSLGKMALIVLGGVAGLLLFIGLGIFFAVSLSKMLKKRSPLTTGVYVKMPPTEPECEKQFQPYFIPINGGGRVKFSRSADAPAYQQGQNQLYNELNLGRREEYDVLDKRRGRDPEMGGKPRRKNPQEGLYNELQKDKMAEAYSEIGMKGERRRGKGHDGLYQGLSTATKDTYDALHMQALPPR

SEQ ID NO: 87 - protein, 654 aa, Homo sapiens
EVQLVESGGGLVKPGGSLKLSCAASGFKFSRYAMSWVRQAPGKRLEWVATISSGGSYIYYPDSVKGRFTISRDNVKNTLYLQMSSLRSEDTAMYYCARRDYDLDYFDSWGQGTLVTVSSGSTSGGGSGGGSGGGGSSDIQMTQSPSSLSASVGDRVTITCKASRDIRSYLTWYQQKPGKAPKTLIYYATSLADGVPSRFSGSGSGQDYSLTISSLESDDTATYYCLQHGESPFTFGSGTKLEIKRAESKYGPPCPPCPAPEFEGGPSVFLFPPKPKDTLMISRTPEVTCVVVDVSQEDPEVQFNWYVDGVEVHNAKTKPREEQFQSTYRVVSVLTVLHQDWLNGKEYKCKVSNKGLPSSIEKTISKAKGQPREPQVYTLPPSQEEMTKNQVSLTCLVKGFYPSDIAVEWESNGQPENNYKTTPPVLDSDGSFFLYSRLTVDKSRWQEGNVFSCSVMHEALHNHYTQKSLSLSLGKMALIVLGGVAGLLLFIGLGIFFKRGRKKLLYIFKQPFMRPVQTTQEEDGCSCRFPEEEEGGCELGGGRVKFSRSADAPAYQQGQNQLYNELNLGRREEYDVLDKRRGRDPEMGGKPRRKNPQEGLYNELQKDKMAEAYSEIGMKGERRRGKGHDGLYQGLSTATKDTYDALHMQALPPR

SEQ ID NO: 88 - protein, 676 aa, Homo sapiens
MLLLVTSLLLCELPHPAFLLIPEVQLVESGGGLVKPGGSLKLSCAASGFKFSRYAMSWVRQAPGKRLEWVATISSGGSYIYYPDSVKGRFTISRDNVKNTLYLQMSSLRSEDTAMYYCARRDYDLDYFDSWGQGTLVTVSSGSTSGGGSGGGSGGGGSSDIQMTQSPSSLSASVGDRVTITCKASRDIRSYLTWYQQKPGKAPKTLIYYATSLADGVPSRFSGSGSGQDYSLTISSLESDDTATYYCLQHGESPFTFGSGTKLEIKRAESKYGPPCPPCPAPEFEGGPSVFLFPPKPKDTLMISRTPEVTCVVVDVSQEDPEVQFNWYVDGVEVHNAKTKPREEQFQSTYRVVSVLTVLHQDWLNGKEYKCKVSNKGLPSSIEKTISKAKGQPREPQVYTLPPSQEEMTKNQVSLTCLVKGFYPSDIAVEWESNGQPENNYKTTPPVLDSDGSFFLYSRLTVDKSRWQEGNVFSCSVMHEALHNHYTQKSLSLSLGKMALIVLGGVAGLLLFIGLGIFFKRGRKKLLYIFKQPFMRPVQTTQEEDGCSCRFPEEEEGGCELGGGRVKFSRSADAPAYQQGQNQLYNELNLGRREEYDVLDKRRGRDPEMGGKPRRKNPQEGLYNELQKDKMAEAYSEIGMKGERRRGKGHDGLYQGLSTATKDTYDALHMQALPPR

SEQ ID NO: 89 - protein, 654 aa, Homo sapiens
DIQMTQSPSSLSASVGDRVTITCKASRDIRSYLTWYQQKPGKAPKTLIYYATSLADGVPSRFSGSGSGQDYSLTISSLESDDTATYYCLQHGESPFTFGSGTKLEIKRAGSTSGGGSGGGSGGGGSSEVQLVESGGGLVKPGGSLKLSCAASGFKFSRYAMSWVRQAPGKRLEWVATISSGGSYIYYPDSVKGRFTISRDNVKNTLYLQMSSLRSEDTAMYYCARRDYDLDYFDSWGQGTLVTVSSESKYGPPCPPCPAPEFEGGPSVFLFPPKPKDTLMISRTPEVTCVVVDVSQEDPEVQFNWYVDGVEVHNAKTKPREEQFQSTYRVVSVLTVLHQDWLNGKEYKCKVSNKGLPSSIEKTISKAKGQPREPQVYTLPPSQEEMTKNQVSLTCLVKGFYPSDIAVEWESNGQPENNYKTTPPVLDSDGSFFLYSRLTVDKSRWQEGNVFSCSVMHEALHNHYTQKSLSLSLGKMALIVLGGVAGLLLFIGLGIFFKRGRKKLLYIFKQPFMRPVQTTQEEDGCSCRFPEEEEGGCELGGGRVKFSRSADAPAYQQGQNQLYNELNLGRREEYDVLDKRRGRDPEMGGKPRRKNPQEGLYNELQKDKMAEAYSEIGMKGERRRGKGHDGLYQGLSTATKDTYDALHMQALPPR

SEQ ID NO: 90 - protein, 676 aa, Homo sapiens
MLLLVTSLLLCELPHPAFLLIPDIQMTQSPSSLSASVGDRVTITCKASRDIRSYLTWYQQKPGKAPKTLIYYATSLADGVPSRFSGSGSGQDYSLTISSLESDDTATYYCLQHGESPFTFGSGTKLEIKRAGSTSGGGSGGGSGGGGSSEVQLVESGGGLVKPGGSLKLSCAASGFKFSRYAMSWVRQAPGKRLEWVATISSGGSYIYYPDSVKGRFTISRDNVKNTLYLQMSSLRSEDTAMYYCARRDYDLDYFDSWGQGTLVTVSSESKYGPPCPPCPAPEFEGGPSVFLFPPKPKDTLMISRTPEVTCVVVDVSQEDPEVQFNWYVDGVEVHNAKTKPREEQFQSTYRVVSVLTVLHQDWLNGKEYKCKVSNKGLPSSIEKTISKAKGQPREPQVYTLPPSQEEMTKNQVSLTCLVKGFYPSDIAVEWESNGQPENNYKTTPPVLDSDGSFFLYSRLTVDKSRWQEGNVFSCSVMHEALHNHYTQKSLSLSLGKMALIVLGGVAGLLLFIGLGIFFKRGRKKLLYIFKQPFMRPVQTTQEEDGCSCRFPEEEEGGCELGGGRVKFSRSADAPAYQQGQNQLYNELNLGRREEYDVLDKRRGRDPEMGGKPRRKNPQEGLYNELQKDKMAEAYSEIGMKGERRRGKGHDGLYQGLSTATKDTYDALHMQALPPR